European Patent Specification EP 3 427 585 B1, published October 16, 2024. Title: Sequence-specific inhbition of small RNA function. Applicant: University of Massachusetts. The sequence listing filed with the application follows.

SEQUENCE LISTING (15 sequences)

SEQ ID NO: 1 - RNA, 31 nt, Artificial Sequence
  synthetic construct
caucacguacgcggaauacuucgaaaugucc

SEQ ID NO: 2 - RNA, 31 nt, Artificial Sequence; identical to SEQ ID NO: 1
  synthetic construct

SEQ ID NO: 3 - RNA, 31 nt, Artificial Sequence
  synthetic construct
ggacauuucgaaguauuccgcguacgugaug

SEQ ID NO: 4 - RNA, 31 nt, Artificial Sequence
  synthetic construct
acauuucgaaguauuccgcguacgugauguu

SEQ ID NO: 5 - RNA, 31 nt, Artificial Sequence
  synthetic construct
ucuucacuauacaaccuacuaccucaaccuu

SEQ ID NO: 6 - RNA, 21 nt, Artificial Sequence
  synthetic construct
uauacaaccuacuaccucauu

SEQ ID NO: 7 - RNA, 34 nt, Artificial Sequence
  synthetic construct
gaacaucacguacgcggaauacuucgaaaugucc

SEQ ID NO: 8 - RNA, 21 nt, Artificial Sequence
  synthetic construct
ucgaaguauuccgcguacgug

SEQ ID NO: 9 - RNA, 21 nt, Artificial Sequence
  synthetic construct
cguacgcggaauacuucgaaa

SEQ ID NO: 10 - RNA, 34 nt, Artificial Sequence
  synthetic construct
ggacauuucgaaguauuccgcguacgugauguuc

SEQ ID NO: 11 - RNA, 36 nt, Artificial Sequence
  synthetic construct
gugaacaucacguacgcggaauacuucgaaaugucc

SEQ ID NO: 12 - RNA, 40 nt, Artificial Sequence
  synthetic construct
ggacauuucgaaguauuccgcguacgugauguucaccucg

SEQ ID NO: 13 - RNA, 21 nt, Artificial Sequence
  synthetic construct
uguacgcggaauacuucgaaa

SEQ ID NO: 14 - RNA, 40 nt, Artificial Sequence
  synthetic construct
ucuucacuauacaaccuacuaccucaaccuuuuauacaac

SEQ ID NO: 15 - RNA, 21 nt, Artificial Sequence
  synthetic construct
ugagguaguagguuguauagu